European Patent Application EP 4 585 604 A1, published July 16, 2025. Title: 核酸の製造方法、不純物の除去方法及び不純物が少ない核酸. Applicant: 株式会社日本触媒. Application JP. The sequence listing filed with the application follows.

SEQUENCE LISTING (2 sequences)

SEQ ID NO: 1 - DNA, 16 bp, Synthetic construct
  source 1..16: mol_type = other DNA
  modified_base 1..16: mod_base = OTHER; note = residues linked by phosphorothioate internucleotide linkages
  modified_base order(1,2,15,16): mod_base = OTHER; note = 2-prime-O,4-prime-C-methylene bridged nucleic acid
  modified_base 16: mod_base = m5c
tgctagcagatgctac

SEQ ID NO: 2 - DNA, 12 bp, synthetic construct
  source 1..12: mol_type = other DNA
  modified_base 1..12: mod_base = OTHER; note = residues linked by phosphorothioate internucleotide linkages
ctagcagatgct